European Patent Application EP 4 737 570 A1, published May 6, 2026. Title: siRNA를 유효성분으로 포함하는 암 예방 또는 치료용 약학적 조성물. Applicant: (주) 엑솔런스. Application KR. The sequence listing filed with the application follows.

SEQUENCE LISTING (66 sequences)

SEQ ID NO: 1 - RNA, 19 nt, synthetic construct
  source 1..19: mol_type = other RNA
gttggagctgatggcgtag

SEQ ID NO: 2 - RNA, 19 nt, synthetic construct
  source 1..19: mol_type = other RNA
agttggagctgatggcgta

SEQ ID NO: 3 - RNA, 19 nt, synthetic construct
  source 1..19: mol_type = other RNA
gttggagctgatggcgtag

SEQ ID NO: 4 - RNA, 19 nt, synthetic construct
  source 1..19: mol_type = other RNA
agttggagctgatggcgta

SEQ ID NO: 5 - RNA, 25 nt, synthetic construct
  source 1..25: mol_type = other RNA
gttggagctgatggcgtaggcaaga

SEQ ID NO: 6 - RNA, 25 nt, synthetic construct
  source 1..25: mol_type = other RNA
gttggagctgatggcgtaggcaaga

SEQ ID NO: 7 - RNA, 25 nt, synthetic construct
  source 1..25: mol_type = other RNA
gttggagctgatggcgtaggcaaga

SEQ ID NO: 8 - RNA, 25 nt, synthetic construct
  source 1..25: mol_type = other RNA
gttggagctgatggcgtaggcaaga

SEQ ID NO: 9 - RNA, 25 nt, synthetic construct
  source 1..25: mol_type = other RNA
gttggagctgatggcgtaggcaaga

SEQ ID NO: 10 - RNA, 25 nt, synthetic construct
  source 1..25: mol_type = other RNA
gttggagctgatggcgtaggcaaga

SEQ ID NO: 11 - RNA, 25 nt, synthetic construct
  source 1..25: mol_type = other RNA
gttggagctgatggcgtagacaaga

SEQ ID NO: 12 - RNA, 25 nt, synthetic construct
  source 1..25: mol_type = other RNA
gttggagctgatggcgtaggcaaga

SEQ ID NO: 13 - RNA, 25 nt, synthetic construct
  source 1..25: mol_type = other RNA
gttggagctgatggcgtaggcaaga

SEQ ID NO: 14 - RNA, 25 nt, synthetic construct
  source 1..25: mol_type = other RNA
gttggagctgatggcgtagacaaga

SEQ ID NO: 15 - RNA, 25 nt, synthetic construct
  source 1..25: mol_type = other RNA
gttggagctgatggcgtagacaaga

SEQ ID NO: 16 - RNA, 25 nt, synthetic construct
  source 1..25: mol_type = other RNA
gttggagctgatggcgtagacaaga

SEQ ID NO: 17 - RNA, 25 nt, synthetic construct
  source 1..25: mol_type = other RNA
gttggagctgatggcgtaggcaaga

SEQ ID NO: 18 - RNA, 25 nt, synthetic construct
  source 1..25: mol_type = other RNA
gttggagctgatggcgtaggcaaga

SEQ ID NO: 19 - RNA, 25 nt, synthetic construct
  source 1..25: mol_type = other RNA
gttggagctgatggcgtaggcaaga

SEQ ID NO: 20 - RNA, 25 nt, synthetic construct
  source 1..25: mol_type = other RNA
gttggagctgatggcgtagacaaga

SEQ ID NO: 21 - RNA, 25 nt, synthetic construct
  source 1..25: mol_type = other RNA
gttggagctgatggcgtagacaaga

SEQ ID NO: 22 - RNA, 25 nt, synthetic construct
  source 1..25: mol_type = other RNA
gttggagctgatggcgtagacaaga

SEQ ID NO: 23 - RNA, 25 nt, synthetic construct
  source 1..25: mol_type = other RNA
gttggagctgatggcgtagtcaaga

SEQ ID NO: 24 - RNA, 25 nt, synthetic construct
  source 1..25: mol_type = other RNA
gttggagctgatggcgtagtcaaga

SEQ ID NO: 25 - RNA, 25 nt, synthetic construct
  source 1..25: mol_type = other RNA
gttggagctgatggcgtagtcaaga

SEQ ID NO: 26 - RNA, 19 nt, synthetic construct
  source 1..19: mol_type = other RNA
agttggagctgatggcgta

SEQ ID NO: 27 - RNA, 19 nt, synthetic construct
  source 1..19: mol_type = other RNA
agttggagctgatggcgta

SEQ ID NO: 28 - RNA, 25 nt, synthetic construct
  source 1..25: mol_type = other RNA
agttggagctgatggcgtaggcaag

SEQ ID NO: 29 - RNA, 25 nt, synthetic construct
  source 1..25: mol_type = other RNA
agttggagctgatggcgtaggcaag

SEQ ID NO: 30 - RNA, 19 nt, synthetic construct
  source 1..19: mol_type = other RNA
ctacgccatcagctccaac

SEQ ID NO: 31 - RNA, 19 nt, synthetic construct
  source 1..19: mol_type = other RNA
tacgccatcagctccaact

SEQ ID NO: 32 - RNA, 19 nt, synthetic construct
  source 1..19: mol_type = other RNA
ctacgccatcagctccaac

SEQ ID NO: 33 - RNA, 19 nt, synthetic construct
  source 1..19: mol_type = other RNA
tacgccatcagctccaact

SEQ ID NO: 34 - RNA, 25 nt, synthetic construct
  source 1..25: mol_type = other RNA
tcttgcctacgccatcagctccaac

SEQ ID NO: 35 - RNA, 25 nt, synthetic construct
  source 1..25: mol_type = other RNA
tcttgcctacgccatcagctccaac

SEQ ID NO: 36 - RNA, 25 nt, synthetic construct
  source 1..25: mol_type = other RNA
tcttgcctacgccatcagctccaac

SEQ ID NO: 37 - RNA, 25 nt, synthetic construct
  source 1..25: mol_type = other RNA
tcttgcctacgccatcagctccaac

SEQ ID NO: 38 - RNA, 25 nt, synthetic construct
  source 1..25: mol_type = other RNA
tcttgcctacgccatcagctccaac

SEQ ID NO: 39 - RNA, 25 nt, synthetic construct
  source 1..25: mol_type = other RNA
tcttgcctacgccatcagctccaac

SEQ ID NO: 40 - RNA, 25 nt, synthetic construct
  source 1..25: mol_type = other RNA
tcttgtctacgccatcagctccaac

SEQ ID NO: 41 - RNA, 25 nt, synthetic construct
  source 1..25: mol_type = other RNA
tcttgcctacgccatcagctccaac

SEQ ID NO: 42 - RNA, 25 nt, synthetic construct
  source 1..25: mol_type = other RNA
tcttgcctacgccatcagctccaac

SEQ ID NO: 43 - RNA, 25 nt, synthetic construct
  source 1..25: mol_type = other RNA
tcttgtctacgccatcagctccaac

SEQ ID NO: 44 - RNA, 25 nt, synthetic construct
  source 1..25: mol_type = other RNA
tcttgtctacgccatcagctccaac

SEQ ID NO: 45 - RNA, 25 nt, synthetic construct
  source 1..25: mol_type = other RNA
tcttgtctacgccatcagctccaac

SEQ ID NO: 46 - RNA, 25 nt, synthetic construct
  source 1..25: mol_type = other RNA
tcttgcctacgccatcagctccaac

SEQ ID NO: 47 - RNA, 25 nt, synthetic construct
  source 1..25: mol_type = other RNA
tcttgcctacgccatcagctccaac

SEQ ID NO: 48 - RNA, 25 nt, synthetic construct
  source 1..25: mol_type = other RNA
tcttgcctacgccatcagctccaac

SEQ ID NO: 49 - RNA, 25 nt, synthetic construct
  source 1..25: mol_type = other RNA
tcttgtctacgccatcagctccaac

SEQ ID NO: 50 - RNA, 25 nt, synthetic construct
  source 1..25: mol_type = other RNA
tcttgtctacgccatcagctccaac

SEQ ID NO: 51 - RNA, 25 nt, synthetic construct
  source 1..25: mol_type = other RNA
tcttgtctacgccatcagctccaac

SEQ ID NO: 52 - RNA, 25 nt, synthetic construct
  source 1..25: mol_type = other RNA
tcttgactacgccatcagctccaac

SEQ ID NO: 53 - RNA, 25 nt, synthetic construct
  source 1..25: mol_type = other RNA
tcttgactacgccatcagctccaac

SEQ ID NO: 54 - RNA, 25 nt, synthetic construct
  source 1..25: mol_type = other RNA
tcttgactacgccatcagctccaac

SEQ ID NO: 55 - RNA, 19 nt, synthetic construct
  source 1..19: mol_type = other RNA
tacgccatcagctccaact

SEQ ID NO: 56 - RNA, 19 nt, synthetic construct
  source 1..19: mol_type = other RNA
tacgccatcagctccaact

SEQ ID NO: 57 - RNA, 25 nt, synthetic construct
  source 1..25: mol_type = other RNA
cttgcctacgccatcagctccaact

SEQ ID NO: 58 - RNA, 25 nt, synthetic construct
  source 1..25: mol_type = other RNA
cttgcctacgccatcagctccaact

SEQ ID NO: 59 - RNA, 19 nt, synthetic construct
  source 1..19: mol_type = other RNA
gttggagctgatggcgtag

SEQ ID NO: 60 - RNA, 19 nt, synthetic construct
  source 1..19: mol_type = other RNA
ctacgccatcagctccaac

SEQ ID NO: 61 - RNA, 19 nt, synthetic construct
  source 1..19: mol_type = other RNA
gaggtgtagggctgtacgt

SEQ ID NO: 62 - RNA, 19 nt, synthetic construct
  source 1..19: mol_type = other RNA
acgtagagccctagacctc

SEQ ID NO: 63 - RNA, 21 nt, synthetic construct
  source 1..21: mol_type = other RNA
gttggagctgatggcgtaggc

SEQ ID NO: 64 - RNA, 21 nt, synthetic construct
  source 1..21: mol_type = other RNA
gcctacgccatcagctccaac

SEQ ID NO: 65 - RNA, 25 nt, synthetic construct
  source 1..25: mol_type = other RNA
gttggagctgatggcgtaggcaaga

SEQ ID NO: 66 - RNA, 25 nt, synthetic construct
  source 1..25: mol_type = other RNA
tcttgcctacgccatcagctccaac